European Patent Specification EP 3 822 349 B1, published December 25, 2024. Title: DNA polymerase variant suitable for nucleic acid amplification reaction from RNA. Applicant: TAKARA BIO INC. The sequence listing filed with the application follows.

SEQUENCE LISTING (27 sequences)

SEQ ID NO: 1 - protein, 834 aa, Thermus thermophilus
MEAMLPLFEPKGRVLLVDGHHLAYRTFFALKGLTTSRGEPVQAVYGFAKSLLKALKEDGYKAVFVVFDAKAPSFRHEAYEAYKAGRAPTPEDFPRQLALIKELVDLLGFTRLEVPGYEADDVLATLAKKAEKEGYEVRILTADRDLYQLVSDRVAVLHPEGHLITPEWLWEKYGLRPEQWVDFRALVGDPSDNLPGVKGIGEKTALKLLKEWGSLENLLKNLDRVKPENVREKIKAHLEDLRLSLELSRVRTDLPLEVDLAQGREPDREGLRAFLERLEFGSLLHEFGLLEAPAPLEEAPWPPPEGAFVGFVLSRPEPMWAELKALAACRDGRVHRAADPLAGLKDLKEVRGLLAKDLAVLASREGLDLVPGDDPMLLAYLLDPSNTTPEGVARRYGGEWTEDAAHRALLSERLHRNLLKRLEGEEKLLWLYHEVEKPLSRVLAHMEATGVRLDVAYLQALSLELAEEIRRLEEEVFRLAGHPFNLNSRDQLERVLFDELRLPALGKTQKTGKRSTSAAVLEALREAHPIVEKILQHRELTKLKNTYVDPLPSLVHPRTGRLHTRFNQTATATGRLSSSDPNLQNIPVRTPLGQRIRRAFVAEAGWALVALDYSQIELRVLAHLSGDENLIRVFQEGKDIHTQTASWMFGVPPEAVDPLMRRAAKTVNFGVLYGMSAHRLSQELAIPYEEAVAFIERYFQSFPKVRAWIEKTLEEGRKRGYVETLFGRRRYVPDLNARVKSVREAAERMAFNMPVQGTAADLMKLAMVKLFPRLREMGARMLLQVHDELLLEAPQARAEEVAALAKEAMEKAYPLAVPLEVEVGMGEDWLSAKG

SEQ ID NO: 2 - DNA, 23 bp, Artificial Sequence
  PCR forward Primer lambda RNA
caggtggcgtattccagattgtc

SEQ ID NO: 3 - DNA, 20 bp, Artificial Sequence
  PCR Reverse Primer lambda RNA
gcaccatactggcaccgaga

SEQ ID NO: 4 - DNA, 18 bp, Artificial Sequence
  Probe lambda RNA. 5'-end is labeled FAM and 3'-end is labeled BHQ1
accaccggccccaatggc

SEQ ID NO: 5 - protein, 834 aa, Artificial Sequence
  DNA polymerase variant Tth b13
MEAMLPLFEPKGRVLLVDGHHLAYRTFFALKGLTTSRGEPVQAVYGFAKSLLKALKEDGYKAVFVVFDAKAPSFRHEAYEAYKAGRAPTPEDFPRQLALIKELVDLLGFTRLEVPGYEADDVLATLAKKAEKEGYEVRILTADRDLYQLVSDRVAVLHPEGHLITPEWLWEKYGLRPEQWVDFRALVGDPSDNLPGVKGIGEKTALKLLKEWGSLENLLKNLDRVKPENVREKIKAHLEDLRLSLELSRVRTDLPLEVDLAQGREPDREGLRAFLERLEFGSLLHEFGLLEAPAPLEEAPWPPPEGAFVGFVLSRPEPMWAELKALAACRDGRVHRAADPLAGLKDLKEVRGLLAKDLAVLASREGLDLVPGDDPMLLAYLLDPSNTTPEGVARRYGGEWTEDAAHRALLSERLHRNLLKRLEGEEKLLWLYHEVEKPLSRVLAHMEATGVRLDVAYLQALSLELAEEIRRLEEEVFRLAGHPFNLNSRDQLERVLFDELRLPALGKTQKTGKRSTSAAVLEALREAHPIVEKILQHRELTKLKNTYVDPLPSLVHPRTGRLHTRFNQTATATGRLSSSDPNLQNIPVRTPLGQRIRRAFVAEAGWALVALDYSQIELRVLAHLSGDENLIRVFQEGKDIHTQTASWMFGVPPEAVDPLMRRAAKTVNFGVLYGMSAHRLSRELAIPYEEAVAFIERYFQSFPKVRAWIEKTLEEGRKRGYVETLFGRRRYVPDLNARVKSVREAAERMAFNMPVQGTAADLMKLAMVKLFPRLREMGARMLLQVHDELLLEAPQARAEEVAALAKEAMEKAYPLAVPLEVEVGMGEDWLSAKG

SEQ ID NO: 6 - DNA, 2505 bp, Artificial Sequence
  DNA polymerase variant Tth b13
atggaagctatgctgccgctgttcgaaccgaaaggtcgtgttctgctggttgacggtcaccacctggcttaccgtaccttcttcgctctgaaaggtctgaccacctctcgtggtgaaccggttcaggctgtttacggtttcgctaaatctctgctgaaagctctgaaagaagatggttacaaagctgttttcgttgtattcgacgcgaaagctccgtctttccgtcacgaagcttacgaagcttacaaagctggtcgtgctccgaccccggaagacttcccgcgtcagctggctctgatcaaagaactggttgacctgctgggtttcacccgtctggaagttccgggttacgaagctgacgacgttctggctaccctggctaaaaaagctgaaaaagaaggttacgaagttcgtatcctgaccgctgaccgtgacctgtaccagctggtttctgaccgtgttgctgttctgcacccggaaggtcacctgatcaccccggaatggctgtgggaaaaatacggtctgcgtccggaacagtgggttgacttccgtgctctggttggtgacccgtctgacaacctgccgggtgttaaaggtatcggtgaaaaaaccgctctgaaactgctgaaagaatggggttctctggaaaacctgctgaaaaacctggaccgtgttaaaccggaaaacgttcgtgaaaaaatcaaagctcacctggaagacctgcgtctgtctctggaactgtctcgtgttcgtaccgacctgccgctggaagttgacctggctcagggtcgtgaaccggaccgtgaaggtctgcgtgctttcctggaacgtctggaattcggttctctgctgcacgaattcggtctgctggaagctccggctccgctggaagaagctccgtggccgcccccggagggtgcgttcgtcggcttcgttctgtctcgtccggaaccgatgtgggctgaactgaaagctctggctgcttgccgtgacggtcgtgttcaccgtgctgctgacccgctggctggtctgaaagacctgaaagaagttcgtggtctgctggctaaagacctggctgttctggcttctcgtgaaggtctggacctggttccgggtgacgacccgatgctgctggcttacctgctggacccgtctaacaccaccccggaaggtgttgctcgtcgttacggtggtgaatggaccgaagacgctgctcaccgtgctctgctgtctgaacgtctgcaccgtaacctgctgaaacgtctggaaggtgaagaaaaactgctgtggctgtaccacgaagttgaaaaaccgctgtctcgtgttctggctcacatggaagctaccggtgttcgtctggacgttgcttacctgcaggctctgtctctggaactggctgaagaaatccgtcgtctggaagaagaagttttccgtctggctggtcacccgttcaacctgaactctcgtgaccagctggaacgtgttctgttcgacgaactgcgtctgccggctctgggtaaaacccagaaaaccggtaaacgttctacctctgctgctgttctggaagctctgcgtgaagctcacccgatcgttgaaaaaatcctgcagcaccgtgaactgaccaaactgaaaaacacctacgttgacccgctgccgtctctggttcacccgcgtaccggtcgtctgcacacccgtttcaaccagaccgctaccgctaccggtcgtctgtcttcttctgacccgaacctgcagaacatcccggttcgtaccccgctgggtcagcgtatccgtcgtgctttcgttgctgaagctggttgggctctggttgctctggactactctcagatcgaactgcgtgttctggctcacctgtctggtgacgaaaacctgatccgtgttttccaggaaggtaaagacatccacacccagaccgcttcttggatgttcggtgttccgccggaagctgttgacccgctgatgcgtcgtgctgctaaaaccgttaacttcggtgttctgtacggtatgtctgctcaccgtctgtctcgtgaactggctatcccgtacgaagaagctgttgctttcatcgaacgttacttccagtctttcccgaaagttcgtgcttggatcgaaaaaaccctggaagaaggtcgtaaacgtggttacgttgaaaccctgttcggtcgtcgtcgttacgttccggacctgaacgctcgtgttaaatctgttcgtgaagctgctgaacgtatggctttcaacatgccggttcagggtaccgctgctgacctgatgaaactggctatggttaaactgttcccgcgtctgcgtgaaatgggtgctcgtatgctgctgcaggttcacgacgaactgctgctggaagctccgcaggctcgtgctgaagaagttgctgctctggctaaagaagctatggaaaaagcttacccgctggctgttccgctggaagttgaagttggtatgggtgaagactggctgtctgctaaaggttaa

SEQ ID NO: 7 - protein, 834 aa, Artificial Sequence
  DNA polymerase variant Tth b46
MEAMLPLFEPKGRVLLVDGHHLAYRTFFALKGLTTSRGEPVQAVYGFAKSLLKALKEDGYKAVFVVFDAKAPSFRHEAYEAYKAGRAPTPEDFPRQLALIKELVDLLGFTRLEVPGYEADDVLATLAKKAEKEGYEVRILTADRDLYQLVSDRVAVLHPEGHLITPEWLWEKYGLRPEQWVDFRALVGDPSDNLPGVKGIGEKTALKLLKEWGSLENLLKNLDRVKPENVREKIKAHLEDLRLSLELSRVRTDLPLEVDLAQGREPDREGLRAFLERLEFGSLLHEFGLLEAPAPLEEAPWPPPEGAFVGFVLSRPEPMWAELKALAACRDGRVHRAADPLAGLKDLKEVRGLLAKDLAVLASREGLDLVPGDDPMLLAYLLDPSNTTPEGVARRYGGEWTEDAAHRALLSERLHRNLLKRLEGEEKLLWLYHEVEKPLSRVLAHMEATGVRLDVAYLQALSLELAEEIRRLEEEVFRLAGHPFNLNSRDQLERVLFDELRLPALGKTQKTGKRSTSAAVLEALREAHPIVEKILQHRELTKLKNTYVDPLPSLVHPRTGRLHTRFNQTATATGRLSSSDPNLQNIPVRTPLGQRIRRAFVAEAGWALVALDYSQIELRVLAHLSGDENLIRVFQEGKDIHTQTASWMFGVPPEAVDPLMRRAAKTVNFGVLYGMSAHRLSQELAIPYREAVAFIERYFQSFPKVRAWIEKTLEEGRKRGYVETLFGRRRYVPDLNARVKSVREAAERMAFNMPVQGTAADLMKLAMVKLFPRLREMGARMLLQVHDELLLEAPQARAEEVAALAKEAMEKAYPLAVPLEVEVGMGEDWLSAKG

SEQ ID NO: 8 - DNA, 2505 bp, Artificial Sequence
  DNA polymerase variant Tth b46
atggaagctatgctgccgctgttcgaaccgaaaggtcgtgttctgctggttgacggtcaccacctggcttaccgtaccttcttcgctctgaaaggtctgaccacctctcgtggtgaaccggttcaggctgtttacggtttcgctaaatctctgctgaaagctctgaaagaagatggttacaaagctgttttcgttgtattcgacgcgaaagctccgtctttccgtcacgaagcttacgaagcttacaaagctggtcgtgctccgaccccggaagacttcccgcgtcagctggctctgatcaaagaactggttgacctgctgggtttcacccgtctggaagttccgggttacgaagctgacgacgttctggctaccctggctaaaaaagctgaaaaagaaggttacgaagttcgtatcctgaccgctgaccgtgacctgtaccagctggtttctgaccgtgttgctgttctgcacccggaaggtcacctgatcaccccggaatggctgtgggaaaaatacggtctgcgtccggaacagtgggttgacttccgtgctctggttggtgacccgtctgacaacctgccgggtgttaaaggtatcggtgaaaaaaccgctctgaaactgctgaaagaatggggttctctggaaaacctgctgaaaaacctggaccgtgttaaaccggaaaacgttcgtgaaaaaatcaaagctcacctggaagacctgcgtctgtctctggaactgtctcgtgttcgtaccgacctgccgctggaagttgacctggctcagggtcgtgaaccggaccgtgaaggtctgcgtgctttcctggaacgtctggaattcggttctctgctgcacgaattcggtctgctggaagctccggctccgctggaagaagctccgtggccgcccccggagggtgcgttcgtcggcttcgttctgtctcgtccggaaccgatgtgggctgaactgaaagctctggctgcttgccgtgacggtcgtgttcaccgtgctgctgacccgctggctggtctgaaagacctgaaagaagttcgtggtctgctggctaaagacctggctgttctggcttctcgtgaaggtctggacctggttccgggtgacgacccgatgctgctggcttacctgctggacccgtctaacaccaccccggaaggtgttgctcgtcgttacggtggtgaatggaccgaagacgctgctcaccgtgctctgctgtctgaacgtctgcaccgtaacctgctgaaacgtctggaaggtgaagaaaaactgctgtggctgtaccacgaagttgaaaaaccgctgtctcgtgttctggctcacatggaagctaccggtgttcgtctggacgttgcttacctgcaggctctgtctctggaactggctgaagaaatccgtcgtctggaagaagaagttttccgtctggctggtcacccgttcaacctgaactctcgtgaccagctggaacgtgttctgttcgacgaactgcgtctgccggctctgggtaaaacccagaaaaccggtaaacgttctacctctgctgctgttctggaagctctgcgtgaagctcacccgatcgttgaaaaaatcctgcagcaccgtgaactgaccaaactgaaaaacacctacgttgacccgctgccgtctctggttcacccgcgtaccggtcgtctgcacacccgtttcaaccagaccgctaccgctaccggtcgtctgtcttcttctgacccgaacctgcagaacatcccggttcgtaccccgctgggtcagcgtatccgtcgtgctttcgttgctgaagctggttgggctctggttgctctggactactctcagatcgaactgcgtgttctggctcacctgtctggtgacgaaaacctgatccgtgttttccaggaaggtaaagacatccacacccagaccgcttcttggatgttcggtgttccgccggaagctgttgacccgctgatgcgtcgtgctgctaaaaccgttaacttcggtgttctgtacggtatgtctgctcaccgtctgtctcaggaactggctatcccgtaccgtgaagctgttgctttcatcgaacgttacttccagtctttcccgaaagttcgtgcttggatcgaaaaaaccctggaagaaggtcgtaaacgtggttacgttgaaaccctgttcggtcgtcgtcgttacgttccggacctgaacgctcgtgttaaatctgttcgtgaagctgctgaacgtatggctttcaacatgccggttcagggtaccgctgctgacctgatgaaactggctatggttaaactgttcccgcgtctgcgtgaaatgggtgctcgtatgctgctgcaggttcacgacgaactgctgctggaagctccgcaggctcgtgctgaagaagttgctgctctggctaaagaagctatggaaaaagcttacccgctggctgttccgctggaagttgaagttggtatgggtgaagactggctgtctgctaaaggttaa

SEQ ID NO: 9 - protein, 834 aa, Artificial Sequence
  DNA polymerase variant Tth b13 b46
MEAMLPLFEPKGRVLLVDGHHLAYRTFFALKGLTTSRGEPVQAVYGFAKSLLKALKEDGYKAVFVVFDAKAPSFRHEAYEAYKAGRAPTPEDFPRQLALIKELVDLLGFTRLEVPGYEADDVLATLAKKAEKEGYEVRILTADRDLYQLVSDRVAVLHPEGHLITPEWLWEKYGLRPEQWVDFRALVGDPSDNLPGVKGIGEKTALKLLKEWGSLENLLKNLDRVKPENVREKIKAHLEDLRLSLELSRVRTDLPLEVDLAQGREPDREGLRAFLERLEFGSLLHEFGLLEAPAPLEEAPWPPPEGAFVGFVLSRPEPMWAELKALAACRDGRVHRAADPLAGLKDLKEVRGLLAKDLAVLASREGLDLVPGDDPMLLAYLLDPSNTTPEGVARRYGGEWTEDAAHRALLSERLHRNLLKRLEGEEKLLWLYHEVEKPLSRVLAHMEATGVRLDVAYLQALSLELAEEIRRLEEEVFRLAGHPFNLNSRDQLERVLFDELRLPALGKTQKTGKRSTSAAVLEALREAHPIVEKILQHRELTKLKNTYVDPLPSLVHPRTGRLHTRFNQTATATGRLSSSDPNLQNIPVRTPLGQRIRRAFVAEAGWALVALDYSQIELRVLAHLSGDENLIRVFQEGKDIHTQTASWMFGVPPEAVDPLMRRAAKTVNFGVLYGMSAHRLSRELAIPYREAVAFIERYFQSFPKVRAWIEKTLEEGRKRGYVETLFGRRRYVPDLNARVKSVREAAERMAFNMPVQGTAADLMKLAMVKLFPRLREMGARMLLQVHDELLLEAPQARAEEVAALAKEAMEKAYPLAVPLEVEVGMGEDWLSAKG

SEQ ID NO: 10 - DNA, 2505 bp, Artificial Sequence
  DNA polymerase variant Tth b13 b46
atggaagctatgctgccgctgttcgaaccgaaaggtcgtgttctgctggttgacggtcaccacctggcttaccgtaccttcttcgctctgaaaggtctgaccacctctcgtggtgaaccggttcaggctgtttacggtttcgctaaatctctgctgaaagctctgaaagaagatggttacaaagctgttttcgttgtattcgacgcgaaagctccgtctttccgtcacgaagcttacgaagcttacaaagctggtcgtgctccgaccccggaagacttcccgcgtcagctggctctgatcaaagaactggttgacctgctgggtttcacccgtctggaagttccgggttacgaagctgacgacgttctggctaccctggctaaaaaagctgaaaaagaaggttacgaagttcgtatcctgaccgctgaccgtgacctgtaccagctggtttctgaccgtgttgctgttctgcacccggaaggtcacctgatcaccccggaatggctgtgggaaaaatacggtctgcgtccggaacagtgggttgacttccgtgctctggttggtgacccgtctgacaacctgccgggtgttaaaggtatcggtgaaaaaaccgctctgaaactgctgaaagaatggggttctctggaaaacctgctgaaaaacctggaccgtgttaaaccggaaaacgttcgtgaaaaaatcaaagctcacctggaagacctgcgtctgtctctggaactgtctcgtgttcgtaccgacctgccgctggaagttgacctggctcagggtcgtgaaccggaccgtgaaggtctgcgtgctttcctggaacgtctggaattcggttctctgctgcacgaattcggtctgctggaagctccggctccgctggaagaagctccgtggccgcccccggagggtgcgttcgtcggcttcgttctgtctcgtccggaaccgatgtgggctgaactgaaagctctggctgcttgccgtgacggtcgtgttcaccgtgctgctgacccgctggctggtctgaaagacctgaaagaagttcgtggtctgctggctaaagacctggctgttctggcttctcgtgaaggtctggacctggttccgggtgacgacccgatgctgctggcttacctgctggacccgtctaacaccaccccggaaggtgttgctcgtcgttacggtggtgaatggaccgaagacgctgctcaccgtgctctgctgtctgaacgtctgcaccgtaacctgctgaaacgtctggaaggtgaagaaaaactgctgtggctgtaccacgaagttgaaaaaccgctgtctcgtgttctggctcacatggaagctaccggtgttcgtctggacgttgcttacctgcaggctctgtctctggaactggctgaagaaatccgtcgtctggaagaagaagttttccgtctggctggtcacccgttcaacctgaactctcgtgaccagctggaacgtgttctgttcgacgaactgcgtctgccggctctgggtaaaacccagaaaaccggtaaacgttctacctctgctgctgttctggaagctctgcgtgaagctcacccgatcgttgaaaaaatcctgcagcaccgtgaactgaccaaactgaaaaacacctacgttgacccgctgccgtctctggttcacccgcgtaccggtcgtctgcacacccgtttcaaccagaccgctaccgctaccggtcgtctgtcttcttctgacccgaacctgcagaacatcccggttcgtaccccgctgggtcagcgtatccgtcgtgctttcgttgctgaagctggttgggctctggttgctctggactactctcagatcgaactgcgtgttctggctcacctgtctggtgacgaaaacctgatccgtgttttccaggaaggtaaagacatccacacccagaccgcttcttggatgttcggtgttccgccggaagctgttgacccgctgatgcgtcgtgctgctaaaaccgttaacttcggtgttctgtacggtatgtctgctcaccgtctgtctcgtgaactggctatcccgtaccgtgaagctgttgctttcatcgaacgttacttccagtctttcccgaaagttcgtgcttggatcgaaaaaaccctggaagaaggtcgtaaacgtggttacgttgaaaccctgttcggtcgtcgtcgttacgttccggacctgaacgctcgtgttaaatctgttcgtgaagctgctgaacgtatggctttcaacatgccggttcagggtaccgctgctgacctgatgaaactggctatggttaaactgttcccgcgtctgcgtgaaatgggtgctcgtatgctgctgcaggttcacgacgaactgctgctggaagctccgcaggctcgtgctgaagaagttgctgctctggctaaagaagctatggaaaaagcttacccgctggctgttccgctggaagttgaagttggtatgggtgaagactggctgtctgctaaaggttaa

SEQ ID NO: 11 - protein, 911 aa, Artificial Sequence
  PIP-L14-PIP-L14-PIP-L15 Tth
MSGKQATLFDFLKSGSGSGSGSGSGSGKQATLFDFLKSGSGSGSGSGSGSGKQATLFDFLKKGSGSGSGSGSGSGSGMEAMLPLFEPKGRVLLVDGHHLAYRTFFALKGLTTSRGEPVQAVYGFAKSLLKALKEDGYKAVFVVFDAKAPSFRHEAYEAYKAGRAPTPEDFPRQLALIKELVDLLGFTRLEVPGYEADDVLATLAKKAEKEGYEVRILTADRDLYQLVSDRVAVLHPEGHLITPEWLWEKYGLRPEQWVDFRALVGDPSDNLPGVKGIGEKTALKLLKEWGSLENLLKNLDRVKPENVREKIKAHLEDLRLSLELSRVRTDLPLEVDLAQGREPDREGLRAFLERLEFGSLLHEFGLLEAPAPLEEAPWPPPEGAFVGFVLSRPEPMWAELKALAACRDGRVHRAADPLAGLKDLKEVRGLLAKDLAVLASREGLDLVPGDDPMLLAYLLDPSNTTPEGVARRYGGEWTEDAAHRALLSERLHRNLLKRLEGEEKLLWLYHEVEKPLSRVLAHMEATGVRLDVAYLQALSLELAEEIRRLEEEVFRLAGHPFNLNSRDQLERVLFDELRLPALGKTQKTGKRSTSAAVLEALREAHPIVEKILQHRELTKLKNTYVDPLPSLVHPRTGRLHTRFNQTATATGRLSSSDPNLQNIPVRTPLGQRIRRAFVAEAGWALVALDYSQIELRVLAHLSGDENLIRVFQEGKDIHTQTASWMFGVPPEAVDPLMRRAAKTVNFGVLYGMSAHRLSQELAIPYEEAVAFIERYFQSFPKVRAWIEKTLEEGRKRGYVETLFGRRRYVPDLNARVKSVREAAERMAFNMPVQGTAADLMKLAMVKLFPRLREMGARMLLQVHDELLLEAPQARAEEVAALAKEAMEKAYPLAVPLEVEVGMGEDWLSAKG

SEQ ID NO: 12 - DNA, 20 bp, Artificial Sequence
  PCR forward Primer COG1F
  misc_feature (12)..(12): n is a, c, g, or t
cgytggatgcgnttycatga

SEQ ID NO: 13 - DNA, 22 bp, Artificial Sequence
  PCR Reverse Primer COG1R
cttagacgccatcatcattyac

SEQ ID NO: 14 - DNA, 26 bp, Artificial Sequence
  PCR forward Primer COG2F
  misc_feature (9)..(9): n is a, c, g, or t
cargarbcnatgttyagrtggatgag

SEQ ID NO: 15 - DNA, 21 bp, Artificial Sequence
  PCR Reverse Primer COG2R
tcgacgccatcttcattcaca

SEQ ID NO: 16 - DNA, 20 bp, Artificial Sequence
  Probe RING1-TP(a). 5'-end is labeled Cy5 and 3'-end is labeled BHQ3
agatygcgatcycctgtcca

SEQ ID NO: 17 - DNA, 20 bp, Artificial Sequence
  Probe RING2AL-TP. 5'end is labeled ROX and 3'-end is labeled BHQ2
tgggagggsgatcgcratct

SEQ ID NO: 18 - protein, 12 aa, Artificial Sequence
  A partial sequence (A1-A12) of  Tth DNA polymerase
LSQELAIPYEEA

SEQ ID NO: 19 - protein, 12 aa, Artificial Sequence
  A partial sequence (A1-A12) of  Tth DNA polymerase variant
LSRELAIPYREA

SEQ ID NO: 20 - protein, 12 aa, Artificial Sequence
  A partial sequence (A1-A12) of Bca polymerase
LAQNLNISRKEA

SEQ ID NO: 21 - protein, 12 aa, Artificial Sequence
  A partial sequence (A1-A12) of Bst polymerase
LAQNLNITRKEA

SEQ ID NO: 22 - protein, 12 aa, Artificial Sequence
  A partial sequence (A1-A12) of Aac polymerase
LAQNLNIPQKEA

SEQ ID NO: 23 - protein, 592 aa, Artificial Sequence
  DNA polymerase I Bacillus caldotenax
MESPSSEEEKPLAKMAFTLADRVTEEMLADKAALVVEVVEENYHDAPIVGIAVVNEHGRFFLRPETALADPQFVAWLGDETKKKSMFDSKRAAVALKWKGIELCGVSFDLLLAAYLLDPAQGVDDVAAAAKMKQYEAVRPDEAVYGKGAKRAVPDEPVLAEHLVRKAAAIWALERPFLDELRRNEQDRLLVELEQPLSSILAEMEFAGVKVDTKRLEQMGEELAEQLRTVEQRIYELAGQEFNINSPKQLGVILFEKLQLPVLKKTKTGYSTSADVLEKLAPYHEIVENILHYRQLGKLQSTYIEGLLKVVRPDTKKVHTIFNQALTQTGRLSSTEPNLQNIPIRLEEGRKIRQAFVPSESDWLIFAADYSQIELRVLAHIAEDDNLMEAFRRDLDIHTKTAMDIFQVSEDEVTPNMRRQAKAVNFGIVYGISDYGLAQNLNISRKEAAEFIERYFESFPGVKRYMENIVQEAKQKGYVTTLLHRRRYLPDITSRNFNVRSFAERMAMNTPIQGSAADIIKKAMIDLNARLKEERLQARLLLQVHDELILEAPKEEMERLCRLVPEVMEQAVTLRVPLKVDYHYGSTWYDAK

SEQ ID NO: 24 - protein, 609 aa, Artificial Sequence
  DNA polymerase I Alicyclobacillus acidocaldarius
MELDFRSLVDKISEEMSHDSTPTPSPAAASGASSEWSSFAYGLIEDAGAWQEAISSFSEPVGVMMDLADPDYHRAEIRGMAVATPKRAYYVRFGERLELSDVRPWLVSDRPKVAFDLKSMAFALDAHGIGLTSECGWQDVKLAAYLLNPQDGEVELSDVFARERGQELPAWEEGEREKWLAYTASQLPPLFESLAYTIRMQEMERLYQEVELPLAFVLAKMEITGFYVNREKLVAFGQELTERIKRITQEIYDLAGTSFNLNSPKQLGEILFDKLGLPALKKTKTGYSTSADVLEKLAPMHEIVQKILDYRLLAKLQSTYVEGLLKVIRKETGRVHTRFHQTLTATGRLSSSEPNLQNIPIRLEEGRRLRQVFEPTYKDWVIFAADYSQIELRILAHLSGDEALIDAFRRDMDIHTRTAADVFEVPPEQVTSLMRRQAKAVNFGIVYGISDFGLAQNLNIPQKEAKRFIESYFEKFPGVKRYMDEIVKQARERGYVTTLMNRRRYLPDIHSRNYQLRSFAERTAMNTPIQGSAADLIKLAMVRIDRAMRDAQMDARMLLQVHDELIFECPKDELAALEVLVRDNMENAMTLSVPLKVDTAYGPTWYDAK

SEQ ID NO: 25 - protein, 832 aa, Artificial Sequence
  DNA polymerase I Thermus aquaticus
MRGMLPLFEPKGRVLLVDGHHLAYRTFHALKGLTTSRGEPVQAVYGFAKSLLKALKEDGDAVIVVFDAKAPSFRHEAYGGYKAGRAPTPEDFPRQLALIKELVDLLGLARLEVPGYEADDVLASLAKKAEKEGYEVRILTADKDLYQLLSDRIHALHPEGYLITPAWLWEKYGLRPDQWADYRALTGDESDNLPGVKGIGEKTARKLLEEWGSLEALLKNLDRLKPAIREKILAHMDDLKLSWDLAKVRTDLPLEVDFAKRREPDRERLRAFLERLEFGSLLHEFGLLESPKALEEAPWPPPEGAFVGFVLSRKEPMWADLLALAAARGGRVHRAPEPYKALRDLKEARGLLAKDLSVLALREGLGLPPGDDPMLLAYLLDPSNTTPEGVARRYGGEWTEEAGERAALSERLFANLWGRLEGEERLLWLYREVERPLSAVLAHMEATGVRLDVAYLRALSLEVAEEIARLEAEVFRLAGHPFNLNSRDQLERVLFDELGLPAIGKTEKTGKRSTSAAVLEALREAHPIVEKILQYRELTKLKSTYIDPLPDLIHPRTGRLHTRFNQTATATGRLSSSDPNLQNIPVRTPLGQRIRRAFIAEEGWLLVALDYSQIELRVLAHLSGDENLIRVFQEGRDIHTETASWMFGVPREAVDPLMRRAAKTINFGVLYGMSAHRLSQELAIPYEEAQAFIERYFQSFPKVRAWIEKTLEEGRRRGYVETLFGRRRYVPDLEARVKSVREAAERMAFNMPVQGTAADLMKLAMVKLFPRLEEMGARMLLQVHDELVLEAPKERAEAVARLAKEVMEGVYPLAVPLEVEVGIGEDWLSAKE

SEQ ID NO: 26 - DNA, 19 bp, Artificial Sequence
  PCR forward Primer hACTB-F
tggcacccagcacaatgaa

SEQ ID NO: 27 - DNA, 20 bp, Artificial Sequence
  PCR Reverse Primer hACTB-533
atcacctcccctgtgtggac